European Patent Specification EP 3 351 548 B1, published August 20, 2025. Title: CROSS-LINKED NUCLEIC ACID GUNA, PREPARATION METHOD OF THE SAME, AND INTERMEDIATE FOR THE SAME. Applicant: Mitsubishi Tanabe Pharma Corporation Osaka University. The sequence listing filed with the application follows.

SEQUENCE LISTING (23 sequences)

SEQ ID NO: 1 - DNA, 10 bp, Artificial Sequence
  Description of Artificial Sequence: oligonucleotide
ttttattttt

SEQ ID NO: 2 - DNA, 10 bp, Artificial Sequence
  Description of Artificial Sequence: oligonucleotide
  modified_base (5)..(5): m5c
ttttnttttt

SEQ ID NO: 3 - DNA, 10 bp, Artificial Sequence
  Description of Artificial Sequence: oligonucleotide
ttttgttttt

SEQ ID NO: 4 - DNA, 12 bp, Artificial Sequence
  Description of Artificial Sequence: oligonucleotide
gcgttttttgct

SEQ ID NO: 5 - DNA, 12 bp, Artificial Sequence
  Description of Artificial Sequence: oligonucleotide
gcgttatttgct

SEQ ID NO: 6 - DNA, 12 bp, Artificial Sequence
  Description of Artificial Sequence: oligonucleotide
  modified_base (6)..(6): m5c
gcgttntttgct

SEQ ID NO: 7 - DNA, 12 bp, Artificial Sequence
  Description of Artificial Sequence: oligonucleotide
gcgttgtttgct

SEQ ID NO: 8 - DNA, 10 bp, Artificial Sequence
  Description of Artificial Sequence: oligonucleotide
tttttttttt

SEQ ID NO: 9 - DNA, 10 bp, Artificial Sequence
  Description of Artificial Sequence: oligonucleotide
aaaaaaaaaa

SEQ ID NO: 10 - DNA, 10 bp, Artificial Sequence
  Description of Artificial Sequence: oligonucleotide
  modified_base (4)..(4): m5c
  modified_base (5)..(5): m5c
  modified_base (6)..(6): m5c
tttnnntttt

SEQ ID NO: 11 - DNA, 10 bp, Artificial Sequence
  Description of Artificial Sequence: oligonucleotide
tttgggtttt

SEQ ID NO: 12 - DNA, 12 bp, Artificial Sequence
  Description of Artificial Sequence: oligonucleotide
agcaaaaaacgc

SEQ ID NO: 13 - RNA, 12 nt, Artificial Sequence
  Description of Artificial Sequence: oligonucleotide
agcaaaaaacgc

SEQ ID NO: 14 - DNA, 12 bp, Artificial Sequence
  Description of Artificial Sequence: oligonucleotide
agcaaataacgc

SEQ ID NO: 15 - RNA, 12 nt, Artificial Sequence
  Description of Artificial Sequence: oligonucleotide
agcaaataacgc

SEQ ID NO: 16 - DNA, 12 bp, Artificial Sequence
  Description of Artificial Sequence: oligonucleotide
agcaaagaacgc

SEQ ID NO: 17 - RNA, 12 nt, Artificial Sequence
  Description of Artificial Sequence: oligonucleotide
agcaaagaacgc

SEQ ID NO: 18 - DNA, 12 bp, Artificial Sequence
  Description of Artificial Sequence: oligonucleotide
agcaaacaacgc

SEQ ID NO: 19 - RNA, 12 nt, Artificial Sequence
  Description of Artificial Sequence: oligonucleotide
agcaaacaacgc

SEQ ID NO: 20 - DNA, 10 bp, Artificial Sequence
  Description of Artificial Sequence: oligonucleotide
aaaaaaaaaa

SEQ ID NO: 21 - DNA, 10 bp, Artificial Sequence
  Description of Artificial Sequence: oligonucleotide
tttttttttt

SEQ ID NO: 22 - DNA, 10 bp, Artificial Sequence
  Description of Artificial Sequence: oligonucleotide
aaaagggaaa

SEQ ID NO: 23 - DNA, 10 bp, Artificial Sequence
  Description of Artificial Sequence: oligonucleotide
aaaacccaaa